European Patent Application EP 4 397 758 A1, published July 10, 2024. Title: Nucleic acid construct capable of measuring homologous recombination activity and use of the same. Applicant: Public University Corporation Yokohama City University. The sequence listing filed with the application follows.

SEQUENCE LISTING (95 sequences)

SEQ ID NO: 1 - DNA, 23 bp, synthetic construct
  misc_feature 1..23: note = primer Nluc-Fw
  source 1..23: mol_type = other DNA
taatacgactcactataggctag

SEQ ID NO: 2 - DNA, 43 bp, synthetic construct
  misc_feature 1..43: note = primer Sce-5'Nluc-Rv
  source 1..43: mol_type = other DNA
attaccctgttatccctatcactggcccatttggtcgccgctc

SEQ ID NO: 3 - DNA, 45 bp, synthetic construct
  misc_feature 1..45: note = primer Sce-3'Nluc-Fw
  source 1..45: mol_type = other DNA
tgatagggataacagggtaatgtgtaccctgtggatgatcatcac

SEQ ID NO: 4 - DNA, 23 bp, synthetic construct
  misc_feature 1..23: note = primer Nluc-Rv
  source 1..23: mol_type = other DNA
ccgccccgactctagagtcgcgg

SEQ ID NO: 5 - DNA, 44 bp, synthetic construct
  misc_feature 1..44: note = primer iNluc-Fw
  source 1..44: mol_type = other DNA
aaatcgataaggatcgctagcatgaagatttcgttggggactgg

SEQ ID NO: 6 - DNA, 44 bp, synthetic construct
  misc_feature 1..44: note = primer iNluc-Rv
  source 1..44: mol_type = other DNA
caccatacgcggatccttatcagttgatggttactcggaacagc

SEQ ID NO: 7 - DNA, 75 bp, synthetic construct
  misc_feature 1..75: note = single-stranded oligonucleotide shRad51-top
  source 1..75: mol_type = other DNA
gatccgcggtcagagatcatacagattctgtgaagccacagatgggaatctgtatgatctctgaccgctttttta

SEQ ID NO: 8 - DNA, 75 bp, synthetic construct
  misc_feature 1..75: note = single-stranded oligonucleotide shRad51-btm
  source 1..75: mol_type = other DNA
agcttaaaaaagcggtcagagatcatacagattcccatctgtggcttcacagaatctgtatgatctctgaccgcg

SEQ ID NO: 9 - DNA, 71 bp, synthetic construct
  misc_feature 1..71: note = single-stranded oligonucleotide shControl-top
  source 1..71: mol_type = other DNA
gatccgcctaaggttaagtcgccctctgtgaagccacagatgggagggcgacttaaccttaggctttttta

SEQ ID NO: 10 - DNA, 71 bp, synthetic construct
  misc_feature 1..71: note = single-stranded oligonucleotide shControl-btm
  source 1..71: mol_type = other DNA
agcttaaaaaagcctaaggttaagtcgccctcccatctgtggcttcacagagggcgacttaaccttaggcg

SEQ ID NO: 11 - DNA, 45 bp, synthetic construct
  misc_feature 1..45: note = primer DTA-Fw
  source 1..45: mol_type = other DNA
actcactataggctagcgtcctcgccatggatcctgatgatgttg

SEQ ID NO: 12 - DNA, 40 bp, synthetic construct
  misc_feature 1..40: note = primer Sce-5'DTA-Rv
  source 1..40: mol_type = other DNA
attaccctgttatccctatcattgtgtaccagattttggc

SEQ ID NO: 13 - DNA, 41 bp, synthetic construct
  misc_feature 1..41: note = primer Sce-3'DTA-Fw
  source 1..41: mol_type = other DNA
tagggataacagggtaataaagggttttatagtaccgacaa

SEQ ID NO: 14 - DNA, 46 bp, synthetic construct
  misc_feature 1..46: note = primer DTA-Rv
  source 1..46: mol_type = other DNA
ccgccccgactctagaatcacaaagatcgcctgacacgatttcctg

SEQ ID NO: 15 - DNA, 42 bp, synthetic construct
  misc_feature 1..42: note = primer iDTA-Fw
  source 1..42: mol_type = other DNA
aaatgtggtaaaatcgatgaattacagctcttaaggctagag

SEQ ID NO: 16 - DNA, 42 bp, synthetic construct
  misc_feature 1..42: note = primer iDTA-Rv
  source 1..42: mol_type = other DNA
acgcggatccttatcgtcagacttgctccatcaacggttcag

SEQ ID NO: 17 - DNA, 26 bp, synthetic construct
  misc_feature 1..26: note = primer Sce-5'TK-Fw
  source 1..26: mol_type = other DNA
cttaatacgactcactataggctagc

SEQ ID NO: 18 - DNA, 44 bp, synthetic construct
  misc_feature 1..44: note = primer Sce-5'TK-Rv
  source 1..44: mol_type = other DNA
ttaccctgttatccctatcagatgggatggcggtcgaagatgag

SEQ ID NO: 19 - DNA, 39 bp, synthetic construct
  misc_feature 1..39: note = primer Sce-3'TK-Fw
  source 1..39: mol_type = other DNA
gatagggataacagggtaatgccgcgcggtaccttatgg

SEQ ID NO: 20 - DNA, 20 bp, synthetic construct
  misc_feature 1..20: note = primer Sce-3'TK-Rv
  source 1..20: mol_type = other DNA
gagtgcaccatacgcggatc

SEQ ID NO: 21 - DNA, 41 bp, synthetic construct
  misc_feature 1..41: note = primer iTK-Fw
  source 1..41: mol_type = other DNA
acatggctcgacagatctatgcgcgtctgcgttcgaccagg

SEQ ID NO: 22 - DNA, 38 bp, synthetic construct
  misc_feature 1..38: note = primer iTK-Rv
  source 1..38: mol_type = other DNA
ggccaatattgaagatctgtcgcatatcgtcggtatgg

SEQ ID NO: 23 - DNA, 516 bp, synthetic construct
  misc_feature 1..516: note = NanoLuc (Nluc) gene encoding modified luciferase
  source 1..516: mol_type = other DNA
  CDS 1..516
atggtcttcacactcgaagatttcgttggggactggcgacagacagccggctacaacctggaccaagtccttgaacagggaggtgtgtccagtttgtttcagaatctcggggtgtccgtaactccgatccaaaggattgtcctgagcggtgaaaatgggctgaagatcgacatccatgtcatcatcccgtatgaaggtctgagcggcgaccaaatgggccagatcgaaaaaatttttaaggtggtgtaccctgtggatgatcatcactttaaggtgatcctgcactatggcacactggtaatcgacggggttacgccgaacatgatcgactatttcggacggccgtatgaaggcatcgccgtgttcgacggcaaaaagatcactgtaacagggaccctgtggaacggcaacaaaattatcgacgagcgcctgatcaaccccgacggctccctgctgttccgagtaaccatcaacggagtgaccggctggcggctgtgcgaacgcattctggcgtaa

SEQ ID NO: 24 - protein, 171 aa, synthetic construct
  REGION 1..171: note = The sequence is a translation of SEQ ID NO: 23.; note = Synthetic Construct
MVFTLEDFVGDWRQTAGYNLDQVLEQGGVSSLFQNLGVSVTPIQRIVLSGENGLKIDIHVIIPYEGLSGDQMGQIEKIFKVVYPVDDHHFKVILHYGTLVIDGVTPNMIDYFGRPYEGIAVFDGKKITVTGTLWNGNKIIDERLINPDGSLLFRVTINGVTGWRLCERILA

SEQ ID NO: 25 - DNA, 516 bp, synthetic construct
  misc_feature 1..516: note = SceNluc fragment
  source 1..516: mol_type = other DNA
  CDS 1..516
atggtcttcacactcgaagatttcgttggggactggcgacagacagccggctacaacctggaccaagtccttgaacagggaggtgtgtccagtttgtttcagaatctcggggtgtccgtaactccgatccaaaggattgtcctgagcggtgaaaatgggctgaagatcgacatccatgtcatcatcccgtatgaaggtctgagcggcgaccaaatgggccagtgatagggataacagggtaatgtgtaccctgtggatgatcatcactttaaggtgatcctgcactatggcacactggtaatcgacggggttacgccgaacatgatcgactatttcggacggccgtatgaaggcatcgccgtgttcgacggcaaaaagatcactgtaacagggaccctgtggaacggcaacaaaattatcgacgagcgcctgatcaaccccgacggctccctgctgttccgagtaaccatcaacggagtgaccggctggcggctgtgcgaacgcattctggcgtaa

SEQ ID NO: 26 - protein, 74 aa, synthetic construct
  REGION 1..74: note = Synthetic Construct
MVFTLEDFVGDWRQTAGYNLDQVLEQGGVSSLFQNLGVSVTPIQRIVLSGENGLKIDIHVIIPYEGLSGDQMGQ

SEQ ID NO: 27 - protein, 93 aa, synthetic construct
  REGION 1..93: note = Synthetic Construct
QGNVYPVDDHHFKVILHYGTLVIDGVTPNMIDYFGRPYEGIAVFDGKKITVTGTLWNGNKIIDERLINPDGSLLFRVTINGVTGWRLCERILA

SEQ ID NO: 28 - DNA, 462 bp, synthetic construct
  misc_feature 1..462: note = iNluc fragment
  source 1..462: mol_type = other DNA
  CDS 1..462: protein_id = 29; translation = EDFVGDWRQTAGYNLDQVLEQGGVSSLFQNLGVSVTPIQRIVLSGENGLKIDIHVIIPYEGLSGDQMGQIEKIFKVVYPVDDHHFKVILHYGTLVIDGVTPNMIDYFGRPYEGIAVFDGKKITVTGTLWNGNKIIDERLINPDGSLLFRVTIN
gaagatttcgttggggactggcgacagacagccggctacaacctggaccaagtccttgaacagggaggtgtgtccagtttgtttcagaatctcggggtgtccgtaactccgatccaaaggattgtcctgagcggtgaaaatgggctgaagatcgacatccatgtcatcatcccgtatgaaggtctgagcggcgaccaaatgggccagatcgaaaaaatttttaaggtggtgtaccctgtggatgatcatcactttaaggtgatcctgcactatggcacactggtaatcgacggggttacgccgaacatgatcgactatttcggacggccgtatgaaggcatcgccgtgttcgacggcaaaaagatcactgtaacagggaccctgtggaacggcaacaaaattatcgacgagcgcctgatcaaccccgacggctccctgctgttccgagtaaccatcaactga

SEQ ID NO: 29 - protein, 153 aa, synthetic construct
EDFVGDWRQTAGYNLDQVLEQGGVSSLFQNLGVSVTPIQRIVLSGENGLKIDIHVIIPYEGLSGDQMGQIEKIFKVVYPVDDHHFKVILHYGTLVIDGVTPNMIDYFGRPYEGIAVFDGKKITVTGTLWNGNKIIDERLINPDGSLLFRVTIN

SEQ ID NO: 30 - DNA, 504 bp, synthetic construct
  misc_feature 1..504: note = iNluc fragmemt amplified by PCR using iNluc-Fw and iNluc-Rv
  source 1..504: mol_type = other DNA
aaatcgataaggatcgctagcatgaagatttcgttggggactggcgacagacagccggctacaacctggaccaagtccttgaacagggaggtgtgtccagtttgtttcagaatctcggggtgtccgtaactccgatccaaaggattgtcctgagcggtgaaaatgggctgaagatcgacatccatgtcatcatcccgtatgaaggtctgagcggcgaccaaatgggccagatcgaaaaaatttttaaggtggtgtaccctgtggatgatcatcactttaaggtgatcctgcactatggcacactggtaatcgacggggttacgccgaacatgatcgactatttcggacggccgtatgaaggcatcgccgtgttcgacggcaaaaagatcactgtaacagggaccctgtggaacggcaacaaaattatcgacgagcgcctgatcaaccccgacggctccctgctgttccgagtaaccatcaactgataaggatccgcgtatggtg

SEQ ID NO: 31 - DNA, 591 bp, Corynebacterium diphtheriae
  source 1..591: mol_type = other DNA
  CDS 1..591: protein_id = 32; translation = MDPDDVVDSSKSFVMENFSSYHGTKPGYVDSIQKGIQKPKSGTQGNYDDDWKGFYSTDNKYDAAGYSVDNENPLSGKAGGVVKVTYPGLTKVLALKVDNAETIKKELGLSLTEPLMEQVGTEEFIKRFGDGASRVVLSLPFAEGSSSVEYINNWEQAKALSVELEINFETRGKRGQDAMYEYMAQACAGNRVRRSL
atggatcctgatgatgttgttgattcttctaaatcttttgtgatggaaaacttttcttcgtaccacgggactaaacctggttatgtagattccattcaaaaaggtatacaaaagccaaaatctggtacacaaggaaattatgacgatgattggaaagggttttatagtaccgacaataaatacgacgctgcgggatactctgtagataatgaaaacccgctctctggaaaagctggaggcgtggtcaaagtgacgtatccaggactgacgaaggttctcgcactaaaagtggataatgccgaaactattaagaaagagttaggtttaagtctcactgaaccgttgatggagcaagtcggaacggaagagtttatcaaaaggttcggtgatggtgcttcgcgtgtagtgctcagccttcccttcgctgaggggagttctagcgttgaatatattaataactgggaacaggcgaaagcgttaagcgtagaacttgagattaattttgaaacccgtggaaaacgtggccaagatgcgatgtatgagtatatggctcaagcctgtgcaggaaatcgtgtcaggcgatctttgtga

SEQ ID NO: 32 - protein, 196 aa, Corynebacterium diphtheriae
MDPDDVVDSSKSFVMENFSSYHGTKPGYVDSIQKGIQKPKSGTQGNYDDDWKGFYSTDNKYDAAGYSVDNENPLSGKAGGVVKVTYPGLTKVLALKVDNAETIKKELGLSLTEPLMEQVGTEEFIKRFGDGASRVVLSLPFAEGSSSVEYINNWEQAKALSVELEINFETRGKRGQDAMYEYMAQACAGNRVRRSL

SEQ ID NO: 33 - DNA, 591 bp, synthetic construct
  misc_feature 1..591: note = SceDTA fragment
  source 1..591: mol_type = other DNA
  CDS 1..591
atggatcctgatgatgttgttgattcttctaaatcttttgtgatggaaaacttttcttcgtaccacgggactaaacctggttatgtagattccattcaaaaaggtatacaaaagccaaaatctggtacacaatgatagggataacagggtaataaagggttttatagtaccgacaataaatacgacgctgcgggatactctgtagataatgaaaacccgctctctggaaaagctggaggcgtggtcaaagtgacgtatccaggactgacgaaggttctcgcactaaaagtggataatgccgaaactattaagaaagagttaggtttaagtctcactgaaccgttgatggagcaagtcggaacggaagagtttatcaaaaggttcggtgatggtgcttcgcgtgtagtgctcagccttcccttcgctgaggggagttctagcgttgaatatattaataactgggaacaggcgaaagcgttaagcgtagaacttgagattaattttgaaacccgtggaaaacgtggccaagatgcgatgtatgagtatatggctcaagcctgtgcaggaaatcgtgtcaggcgatctttgtga

SEQ ID NO: 34 - protein, 44 aa, synthetic construct
  REGION 1..44: note = Synthetic Construct
MDPDDVVDSSKSFVMENFSSYHGTKPGYVDSIQKGIQKPKSGTQ

SEQ ID NO: 35 - protein, 148 aa, synthetic construct
  REGION 1..148: note = The sequence is a translation of 145-591nt of SEQ ID NO:33.; note = Synthetic Construct
QGNKGFYSTDNKYDAAGYSVDNENPLSGKAGGVVKVTYPGLTKVLALKVDNAETIKKELGLSLTEPLMEQVGTEEFIKRFGDGASRVVLSLPFAEGSSSVEYINNWEQAKALSVELEINFETRGKRGQDAMYEYMAQACAGNRVRRSL

SEQ ID NO: 36 - DNA, 360 bp, synthetic construct
  misc_feature 1..360: note = partial region of iDTA fragment
  source 1..360: mol_type = other DNA
  CDS 1..360
atggatcctgatgatgttgttgattcttctaaatcttttgtgatggaaaacttttcttcgtaccacgggactaaacctggttatgtagattccattcaaaaaggtatacaaaagccaaaatctggtacacaaggaaattatgacgatgattggaaagggttttatagtaccgacaataaatacgacgctgcgggatactctgtagataatgaaaacccgctctctggaaaagctggaggcgtggtcaaagtgacgtatccaggactgacgaaggttctcgcactaaaagtggataatgccgaaactattaagaaagagttaggtttaagtctcactgaaccgttgatggagcaagtctga

SEQ ID NO: 37 - protein, 119 aa, synthetic construct
  REGION 1..119: note = Synthetic Construct; note = The sequence is a translation of SEQ ID NO: 36.
MDPDDVVDSSKSFVMENFSSYHGTKPGYVDSIQKGIQKPKSGTQGNYDDDWKGFYSTDNKYDAAGYSVDNENPLSGKAGGVVKVTYPGLTKVLALKVDNAETIKKELGLSLTEPLMEQV

SEQ ID NO: 38 - DNA, 1131 bp, herpes simplex virus
  source 1..1131: mol_type = other DNA
  CDS 1..1131
atggcttcgtaccccggccatcaacacgcgtctgcgttcgaccaggctgcgcgttctcgcggccatagcaaccgacgtacggcgttgcgccctcgccggcagcaagaagccacggaagtccgcccggagcagaaaatgcccacgctactgcgggtttatatagacggtccccacgggatggggaaaaccaccaccacgcaactgctggtggccctgggttcgcgcgacgatatcgtctacgtacccgagccgatgacttactggcgggtgctgggggcttccgagacaatcgcgaacatctacaccacacaacaccgcctcgaccagggtgagatatcggccggggacgcggcggtggtaatgacaagcgcccagataacaatgggcatgccttatgccgtgaccgacgccgttctggctcctcatatcgggggggaggctgggagctcacatgccccgcccccggccctcaccctcatcttcgaccgccatcccatcgccgccctcctgtgctacccggccgcgcggtaccttatgggcagcatgaccccccaggccgtgctggcgttcgtggccctcatcccgccgaccttgcccggcaccaacatcgtgcttggggcccttccggaggacagacacatcgaccgcctggccaaacgccagcgccccggcgagcggctggacctggctatgctggctgcgattcgccgcgtttacgggctacttgccaatacggtgcggtatctgcagtgcggcgggtcgtggcgggaggactggggacagctttcggggacggccgtgccgccccagggtgccgagccccagagcaacgcgggcccacgaccccatatcggggacacgttatttaccctgtttcgggcccccgagttgctggcccccaacggcgacctgtataacgtgtttgcctgggccttggacgtcttggccaaacgcctccgttccatgcacgtctttatcctggattacgaccaatcgcccgccggctgccgggacgccctgctgcaacttacctccgggatggtccagacccacgtcaccacccccggctccataccgacgatatgcgacctggcgcgcacgtttgcccgggagatgggggaggctaactga

SEQ ID NO: 39 - protein, 376 aa, herpes simplex virus
  source 1..376: note = The sequence is a translation of SEQ ID NO: 38.
MASYPGHQHASAFDQAARSRGHSNRRTALRPRRQQEATEVRPEQKMPTLLRVYIDGPHGMGKTTTTQLLVALGSRDDIVYVPEPMTYWRVLGASETIANIYTTQHRLDQGEISAGDAAVVMTSAQITMGMPYAVTDAVLAPHIGGEAGSSHAPPPALTLIFDRHPIAALLCYPAARYLMGSMTPQAVLAFVALIPPTLPGTNIVLGALPEDRHIDRLAKRQRPGERLDLAMLAAIRRVYGLLANTVRYLQCGGSWREDWGQLSGTAVPPQGAEPQSNAGPRPHIGDTLFTLFRAPELLAPNGDLYNVFAWALDVLAKRLRSMHVFILDYDQSPAGCRDALLQLTSGMVQTHVTTPGSIPTICDLARTFAREMGEAN

SEQ ID NO: 40 - DNA, 1131 bp, synthetic construct
  misc_feature 1..1131: note = SceTK fragment
  source 1..1131: mol_type = other DNA
  CDS 1..1131
atggcttcgtaccccggccatcaacacgcgtctgcgttcgaccaggctgcgcgttctcgcggccatagcaaccgacgtacggcgttgcgccctcgccggcagcaagaagccacggaagtccgcccggagcagaaaatgcccacgctactgcgggtttatatagacggtccccacgggatggggaaaaccaccaccacgcaactgctggtggccctgggttcgcgcgacgatatcgtctacgtacccgagccgatgacttactggcgggtgctgggggcttccgagacaatcgcgaacatctacaccacacaacaccgcctcgaccagggtgagatatcggccggggacgcggcggtggtaatgacaagcgcccagataacaatgggcatgccttatgccgtgaccgacgccgttctggctcctcatatcgggggggaggctgggagctcacatgccccgcccccggccctcaccctcatcttcgaccgccatcccatctgatagggataacagggtaatgccgcgcggtaccttatgggcagcatgaccccccaggccgtgctggcgttcgtggccctcatcccgccgaccttgcccggcaccaacatcgtgcttggggcccttccggaggacagacacatcgaccgcctggccaaacgccagcgccccggcgagcggctggacctggctatgctggctgcgattcgccgcgtttacgggctacttgccaatacggtgcggtatctgcagtgcggcgggtcgtggcgggaggactggggacagctttcggggacggccgtgccgccccagggtgccgagccccagagcaacgcgggcccacgaccccatatcggggacacgttatttaccctgtttcgggcccccgagttgctggcccccaacggcgacctgtataacgtgtttgcctgggccttggacgtcttggccaaacgcctccgttccatgcacgtctttatcctggattacgaccaatcgcccgccggctgccgggacgccctgctgcaacttacctccgggatggtccagacccacgtcaccacccccggctccataccgacgatatgcgacctggcgcgcacgtttgcccgggagatgggggaggctaactga

SEQ ID NO: 41 - protein, 166 aa, synthetic construct
  REGION 1..166: note = Synthetic Construct
MASYPGHQHASAFDQAARSRGHSNRRTALRPRRQQEATEVRPEQKMPTLLRVYIDGPHGMGKTTTTQLLVALGSRDDIVYVPEPMTYWRVLGASETIANIYTTQHRLDQGEISAGDAAVVMTSAQITMGMPYAVTDAVLAPHIGGEAGSSHAPPPALTLIFDRHPI

SEQ ID NO: 42 - protein, 206 aa, synthetic construct
  REGION 1..206: note = Synthetic Construct
QGNAARYLMGSMTPQAVLAFVALIPPTLPGTNIVLGALPEDRHIDRLAKRQRPGERLDLAMLAAIRRVYGLLANTVRYLQCGGSWREDWGQLSGTAVPPQGAEPQSNAGPRPHIGDTLFTLFRAPELLAPNGDLYNVFAWALDVLAKRLRSMHVFILDYDQSPAGCRDALLQLTSGMVQTHVTTPGSIPTICDLARTFAREMGEAN

SEQ ID NO: 43 - DNA, 1063 bp, synthetic construct
  misc_feature 1..1063: note = iTK fragment
  source 1..1063: mol_type = other DNA
  CDS 2..1063
cgcgtctgcgttcgaccaggctgcgcgttctcgcggccatagcaaccgacgtacggcgttgcgccctcgccggcagcaagaagccacggaagtccgcccggagcagaaaatgcccacgctactgcgggtttatatagacggtccccacgggatggggaaaaccaccaccacgcaactgctggtggccctgggttcgcgcgacgatatcgtctacgtacccgagccgatgacttactggcgggtgctgggggcttccgagacaatcgcgaacatctacaccacacaacaccgcctcgaccagggtgagatatcggccggggacgcggcggtggtaatgacaagcgcccagataacaatgggcatgccttatgccgtgaccgacgccgttctggctcctcatatcgggggggaggctgggagctcacatgccccgcccccggccctcaccctcatcttcgaccgccatcccatcgccgccctcctgtgctacccggccgcgcggtaccttatgggcagcatgaccccccaggccgtgctggcgttcgtggccctcatcccgccgaccttgcccggcaccaacatcgtgcttggggcccttccggaggacagacacatcgaccgcctggccaaacgccagcgccccggcgagcggctggacctggctatgctggctgcgattcgccgcgtttacgggctacttgccaatacggtgcggtatctgcagtgcggcgggtcgtggcgggaggactggggacagctttcggggacggccgtgccgccccagggtgccgagccccagagcaacgcgggcccacgaccccatatcggggacacgttatttaccctgtttcgggcccccgagttgctggcccccaacggcgacctgtataacgtgtttgcctgggccttggacgtcttggccaaacgcctccgttccatgcacgtctttatcctggattacgaccaatcgcccgccggctgccgggacgccctgctgcaacttacctccgggatggtccagacccacgtcaccacccccggctccataccgacgatatgcgac

SEQ ID NO: 44 - protein, 354 aa, synthetic construct
  REGION 1..354: note = Synthetic Construct; note = The sequence is a translation of 2-1063nt of SEQ ID NO: 43.
ASAFDQAARSRGHSNRRTALRPRRQQEATEVRPEQKMPTLLRVYIDGPHGMGKTTTTQLLVALGSRDDIVYVPEPMTYWRVLGASETIANIYTTQHRLDQGEISAGDAAVVMTSAQITMGMPYAVTDAVLAPHIGGEAGSSHAPPPALTLIFDRHPIAALLCYPAARYLMGSMTPQAVLAFVALIPPTLPGTNIVLGALPEDRHIDRLAKRQRPGERLDLAMLAAIRRVYGLLANTVRYLQCGGSWREDWGQLSGTAVPPQGAEPQSNAGPRPHIGDTLFTLFRAPELLAPNGDLYNVFAWALDVLAKRLRSMHVFILDYDQSPAGCRDALLQLTSGMVQTHVTTPGSIPTICD

SEQ ID NO: 45 - DNA, 420 bp, synthetic construct
  misc_feature 1..420: note = iDTA fragment
  source 1..420: mol_type = other DNA
aattacagctcttaaggctagagtacttaatacgactcactataggctagcgtcctcgccatggatcctgatgatgttgttgattcttctaaatcttttgtgatggaaaacttttcttcgtaccacgggactaaacctggttatgtagattccattcaaaaaggtatacaaaagccaaaatctggtacacaaggaaattatgacgatgattggaaagggttttatagtaccgacaataaatacgacgctgcgggatactctgtagataatgaaaacccgctctctggaaaagctggaggcgtggtcaaagtgacgtatccaggactgacgaaggttctcgcactaaaagtggataatgccgaaactattaagaaagagttaggtttaagtctcactgaaccgttgatggagcaagtctga

SEQ ID NO: 46 - DNA, 1131 bp, synthetic construct
  source 1..1131: mol_type = other DNA
  CDS 1..1131: protein_id = 47; translation = MASYPGHQHASAFDQAARSRGHSNRRTALRPRRQQEATEVRPEQKMPTLLRVYIDGPHGMGKTTTTQLLVALGSRDDIVYVPEPMTYWRVLGASETIANIYTTQHRLDQGEISAGDAAVVMTSAQITMGMPYAVTDAVLAPHIGGEAGSSHVPPPALTILADRHPIAYFLCYPAARYLMGSMTPQAVLAFVALIPPTLPGTNIVLGALPEDRHIDRLAKRQRPGERLDLAMLAAIRRVYGLLANTVRYLQCGGSWREDWGQLSGTAVPPQGAEPQSNAGPRPHIGDTLFTLFRAPELLAPNGDLYNVFAWALDVLAKRLRSMHVFILDYDQSPAGCRDALLQLTSGMVQTHVTTPGSIPTICDLARTFAREMGEAN
atggcttcgtaccccggccatcaacacgcgtctgcgttcgaccaggctgcgcgttctcgcggccatagcaaccgacgtacggcgttgcgccctcgccggcagcaagaagccacggaagtccgcccggagcagaaaatgcccacgctactgcgggtttatatagacggtccccacgggatggggaaaaccaccaccacgcaactgctggtggccctgggttcgcgcgacgatatcgtctacgtacccgagccgatgacttactggcgggtgctgggggcttccgagacaatcgcgaacatctacaccacacaacaccgcctcgaccagggtgagatatcggccggggacgcggcggtggtaatgacaagcgcccagataacaatgggcatgccttatgccgtgaccgacgccgttctggctcctcatatcgggggggaggctgggagctcacatgtgccgcccccggccctcaccatcctggccgaccgccatcccatcgcctacttcctgtgctacccggccgcgcggtaccttatgggcagcatgaccccccaggccgtgctggcgttcgtggccctcatcccgccgaccttgcccggcaccaacatcgtgcttggggcccttccggaggacagacacatcgaccgcctggccaaacgccagcgccccggcgagcggctggacctggctatgctggctgcgattcgccgcgtttacgggctacttgccaatacggtgcggtatctgcagtgcggcgggtcgtggcgggaggactggggacagctttcggggacggccgtgccgccccagggtgccgagccccagagcaacgcgggcccacgaccccatatcggggacacgttatttaccctgtttcgggcccccgagttgctggcccccaacggcgacctgtataacgtgtttgcctgggccttggacgtcttggccaaacgcctccgttccatgcacgtctttatcctggattacgaccaatcgcccgccggctgccgggacgccctgctgcaacttacctccgggatggtccagacccacgtcaccacccccggctccataccgacgatatgcgacctggcgcgcacgtttgcccgggagatgggggaggctaactga

SEQ ID NO: 47 - protein, 376 aa, synthetic construct
MASYPGHQHASAFDQAARSRGHSNRRTALRPRRQQEATEVRPEQKMPTLLRVYIDGPHGMGKTTTTQLLVALGSRDDIVYVPEPMTYWRVLGASETIANIYTTQHRLDQGEISAGDAAVVMTSAQITMGMPYAVTDAVLAPHIGGEAGSSHVPPPALTILADRHPIAYFLCYPAARYLMGSMTPQAVLAFVALIPPTLPGTNIVLGALPEDRHIDRLAKRQRPGERLDLAMLAAIRRVYGLLANTVRYLQCGGSWREDWGQLSGTAVPPQGAEPQSNAGPRPHIGDTLFTLFRAPELLAPNGDLYNVFAWALDVLAKRLRSMHVFILDYDQSPAGCRDALLQLTSGMVQTHVTTPGSIPTICDLARTFAREMGEAN

SEQ ID NO: 48 - DNA, 1063 bp, synthetic construct
  source 1..1063: mol_type = other DNA
  CDS 2..1063: protein_id = 49; translation = ASAFDQAARSRGHSNRRTALRPRRQQEATEVRPEQKMPTLLRVYIDGPHGMGKTTTTQLLVALGSRDDIVYVPEPMTYWRVLGASETIANIYTTQHRLDQGEISAGDAAVVMTSAQITMGMPYAVTDAVLAPHIGGEAGSSHVPPPALTILADRHPIAYFLCYPAARYLMGSMTPQAVLAFVALIPPTLPGTNIVLGALPEDRHIDRLAKRQRPGERLDLAMLAAIRRVYGLLANTVRYLQCGGSWREDWGQLSGTAVPPQGAEPQSNAGPRPHIGDTLFTLFRAPELLAPNGDLYNVFAWALDVLAKRLRSMHVFILDYDQSPAGCRDALLQLTSGMVQTHVTTPGSIPTICD
cgcgtctgcgttcgaccaggctgcgcgttctcgcggccatagcaaccgacgtacggcgttgcgccctcgccggcagcaagaagccacggaagtccgcccggagcagaaaatgcccacgctactgcgggtttatatagacggtccccacgggatggggaaaaccaccaccacgcaactgctggtggccctgggttcgcgcgacgatatcgtctacgtacccgagccgatgacttactggcgggtgctgggggcttccgagacaatcgcgaacatctacaccacacaacaccgcctcgaccagggtgagatatcggccggggacgcggcggtggtaatgacaagcgcccagataacaatgggcatgccttatgccgtgaccgacgccgttctggctcctcatatcgggggggaggctgggagctcacatgtgccgcccccggccctcaccatcctggccgaccgccatcccatcgcctacttcctgtgctacccggccgcgcggtaccttatgggcagcatgaccccccaggccgtgctggcgttcgtggccctcatcccgccgaccttgcccggcaccaacatcgtgcttggggcccttccggaggacagacacatcgaccgcctggccaaacgccagcgccccggcgagcggctggacctggctatgctggctgcgattcgccgcgtttacgggctacttgccaatacggtgcggtatctgcagtgcggcgggtcgtggcgggaggactggggacagctttcggggacggccgtgccgccccagggtgccgagccccagagcaacgcgggcccacgaccccatatcggggacacgttatttaccctgtttcgggcccccgagttgctggcccccaacggcgacctgtataacgtgtttgcctgggccttggacgtcttggccaaacgcctccgttccatgcacgtctttatcctggattacgaccaatcgcccgccggctgccgggacgccctgctgcaacttacctccgggatggtccagacccacgtcaccacccccggctccataccgacgatatgcgac

SEQ ID NO: 49 - protein, 354 aa, synthetic construct
ASAFDQAARSRGHSNRRTALRPRRQQEATEVRPEQKMPTLLRVYIDGPHGMGKTTTTQLLVALGSRDDIVYVPEPMTYWRVLGASETIANIYTTQHRLDQGEISAGDAAVVMTSAQITMGMPYAVTDAVLAPHIGGEAGSSHVPPPALTILADRHPIAYFLCYPAARYLMGSMTPQAVLAFVALIPPTLPGTNIVLGALPEDRHIDRLAKRQRPGERLDLAMLAAIRRVYGLLANTVRYLQCGGSWREDWGQLSGTAVPPQGAEPQSNAGPRPHIGDTLFTLFRAPELLAPNGDLYNVFAWALDVLAKRLRSMHVFILDYDQSPAGCRDALLQLTSGMVQTHVTTPGSIPTICD

SEQ ID NO: 50 - DNA, 1122 bp, synthetic construct
  source 1..1122: mol_type = other DNA
  CDS 1..1122: protein_id = 51; translation = MVTGGMASKWDQKGMDIAYEEAALGYKEGGVPIGGCLINNKDGSVLGRGHNMRFQKGSATLHGEISTLENCGRLEGKVYKDTTLYTTLSPCDMCTGAIIMYGIPRCVVGENVNFKSKGEKYLQTRGHEVVVVDDERCKKIMKQFIDERPQDWFEDIGEASEPFKNVYLLPQTNQLLGLYTIIRNKNTTRPDFIFYSDRIIRLLVEEGLNHLPVQKQIVETDTNENFEGVSFMGKICGVSIVRAGESMEQGLRDCCRSVRIGKILIQRDEETALPKLFYEKLPEDISERYVFLLDPMLATGGSAIMATEVLIKRGVKPERIYFLNLICSKEGIEKYHAAFPEVRIVTGALDRGLDENKYLVPGLGDFGDRYYCV
atggtcacaggaggcatggcttcaaagtgggaccagaagggcatggacattgcctatgaggaggctgctctgggctacaaggagggaggggtcccaattggtggctgcctcatcaacaacaaggatggcagtgtcctgggcaggggccacaacatgaggttccagaagggcagtgccaccctgcatggggagatcagcaccctggagaactgtggcaggctggagggcaaggtctacaaggacaccactctgtacaccaccctcagcccttgtgacatgtgcacaggggccatcatcatgtatggcattcccaggtgtgtggtgggagagaatgtcaacttcaagtcaaaaggagagaagtacctccagaccaggggccatgaggtggttgtggtggatgatgagaggtgcaagaagattatgaagcagttcattgatgagagaccccaggactggtttgaggacattggggaggcctctgagcccttcaagaatgtgtacctcctcccccagaccaaccaactcctgggactctacaccatcatcaggaacaagaacaccaccaggccagacttcatcttctacagtgacaggatcatcaggctcctggtggaggagggcctcaaccacctccctgtgcagaagcagattgtggagactgacaccaatgagaactttgagggagtgtctttcatgggcaagatttgtggggtgtccattgtgagggctggggagagcatggagcagggcctgagggactgttgcaggagtgtgaggattggcaagatcctgatccagagggatgaggagactgccctgcccaagctgttctatgagaagctccctgaagacatctctgagaggtatgtcttcctcctggaccccatgctggcaactggaggctctgcaatcatggccactgaggtgctcatcaagaggggagtcaagcctgagaggatctacttcctcaacctcatctgctcaaaggagggcattgagaagtaccatgctgccttccctgaagtgaggattgtcactggggctctggacaggggcctggatgagaacaagtacctggtccctggcctgggagactttggggacagatactactgtgtctaa

SEQ ID NO: 51 - protein, 373 aa, synthetic construct
MVTGGMASKWDQKGMDIAYEEAALGYKEGGVPIGGCLINNKDGSVLGRGHNMRFQKGSATLHGEISTLENCGRLEGKVYKDTTLYTTLSPCDMCTGAIIMYGIPRCVVGENVNFKSKGEKYLQTRGHEVVVVDDERCKKIMKQFIDERPQDWFEDIGEASEPFKNVYLLPQTNQLLGLYTIIRNKNTTRPDFIFYSDRIIRLLVEEGLNHLPVQKQIVETDTNENFEGVSFMGKICGVSIVRAGESMEQGLRDCCRSVRIGKILIQRDEETALPKLFYEKLPEDISERYVFLLDPMLATGGSAIMATEVLIKRGVKPERIYFLNLICSKEGIEKYHAAFPEVRIVTGALDRGLDENKYLVPGLGDFGDRYYCV

SEQ ID NO: 52 - DNA, 477 bp, synthetic construct
  source 1..477: mol_type = other DNA
  CDS 1..477: protein_id = 53; translation = MVTGGMASKWDQKGMDIAYEEAALGYKEGGVPIGGCLINNKDGSVLGRGHNMRFQKGSATLHGEISTLENCGRLEGKVYKDTTLYTTLSPCDMCTGAIIMYGIPRCVVGENVNFKSKGEKYLQTRGHEVVVVDDERCKKIMKQFIDERPQDWFEDIGE
atggtcacaggaggcatggcttcaaagtgggaccagaagggcatggacattgcctatgaggaggctgctctgggctacaaggagggaggggtcccaattggtggctgcctcatcaacaacaaggatggcagtgtcctgggcaggggccacaacatgaggttccagaagggcagtgccaccctgcatggggagatcagcaccctggagaactgtggcaggctggagggcaaggtctacaaggacaccactctgtacaccaccctcagcccttgtgacatgtgcacaggggccatcatcatgtatggcattcccaggtgtgtggtgggagagaatgtcaacttcaagtcaaaaggagagaagtacctccagaccaggggccatgaggtggttgtggtggatgatgagaggtgcaagaagattatgaagcagttcattgatgagagaccccaggactggtttgaggacattggggagtga

SEQ ID NO: 53 - protein, 158 aa, synthetic construct
MVTGGMASKWDQKGMDIAYEEAALGYKEGGVPIGGCLINNKDGSVLGRGHNMRFQKGSATLHGEISTLENCGRLEGKVYKDTTLYTTLSPCDMCTGAIIMYGIPRCVVGENVNFKSKGEKYLQTRGHEVVVVDDERCKKIMKQFIDERPQDWFEDIGE

SEQ ID NO: 54 - DNA, 651 bp, synthetic construct
  source 1..651: mol_type = other DNA
  CDS 1..651: protein_id = 55; translation = MSSEPFKNVYLLPQTNQLLGLYTIIRNKNTTRPDFIFYSDRIIRLLVEEGLNHLPVQKQIVETDTNENFEGVSFMGKICGVSIVRAGESMEQGLRDCCRSVRIGKILIQRDEETALPKLFYEKLPEDISERYVFLLDPMLATGGSAIMATEVLIKRGVKPERIYFLNLICSKEGIEKYHAAFPEVRIVTGALDRGLDENKYLVPGLGDFGDRYYCV
atgtcctctgagcccttcaagaatgtgtacctcctcccccagaccaaccaactcctgggactctacaccatcatcaggaacaagaacaccaccaggccagacttcatcttctacagtgacaggatcatcaggctcctggtggaggagggcctcaaccacctccctgtgcagaagcagattgtggagactgacaccaatgagaactttgagggagtgtctttcatgggcaagatttgtggggtgtccattgtgagggctggggagagcatggagcagggcctgagggactgttgcaggagtgtgaggattggcaagatcctgatccagagggatgaggagactgccctgcccaagctgttctatgagaagctccctgaagacatctctgagaggtatgtcttcctcctggaccccatgctggcaactggaggctctgcaatcatggccactgaggtgctcatcaagaggggagtcaagcctgagaggatctacttcctcaacctcatctgctcaaaggagggcattgagaagtaccatgctgccttccctgaagtgaggattgtcactggggctctggacaggggcctggatgagaacaagtacctggtccctggcctgggagactttggggacagatactactgtgtctaa

SEQ ID NO: 55 - protein, 216 aa, synthetic construct
MSSEPFKNVYLLPQTNQLLGLYTIIRNKNTTRPDFIFYSDRIIRLLVEEGLNHLPVQKQIVETDTNENFEGVSFMGKICGVSIVRAGESMEQGLRDCCRSVRIGKILIQRDEETALPKLFYEKLPEDISERYVFLLDPMLATGGSAIMATEVLIKRGVKPERIYFLNLICSKEGIEKYHAAFPEVRIVTGALDRGLDENKYLVPGLGDFGDRYYCV

SEQ ID NO: 56 - DNA, 1120 bp, synthetic construct
  source 1..1120: mol_type = other DNA
  CDS 1..270: protein_id = 57; translation = MVTGGMASKWDQKGMDIAYEEAALGYKEGGVPIGGCLINNKDGSVLGRGHNMRFQKGSATLHGEISTLENCGRLEGKVYKDTTLYTTLSP
atggtcacaggaggcatggcttcaaagtgggaccagaagggcatggacattgcctatgaggaggctgctctgggctacaaggagggaggggtcccaattggtggctgcctcatcaacaacaaggatggcagtgtcctgggcaggggccacaacatgaggttccagaagggcagtgccaccctgcatggggagatcagcaccctggagaactgtggcaggctggagggcaaggtctacaaggacaccactctgtacaccaccctcagcccttgacgcgtagggataacagggtaatgcatatggcattcccaggtgtgtggtgggagagaatgtcaacttcaagtcaaaaggagagaagtacctccagaccaggggccatgaggtggttgtggtggatgatgagaggtgcaagaagattatgaagcagttcattgatgagagaccccaggactggtttgaggacattggggaggcctctgagcccttcaagaatgtgtacctcctcccccagaccaaccaactcctgggactctacaccatcatcaggaacaagaacaccaccaggccagacttcatcttctacagtgacaggatcatcaggctcctggtggaggagggcctcaaccacctccctgtgcagaagcagattgtggagactgacaccaatgagaactttgagggagtgtctttcatgggcaagatttgtggggtgtccattgtgagggctggggagagcatggagcagggcctgagggactgttgcaggagtgtgaggattggcaagatcctgatccagagggatgaggagactgccctgcccaagctgttctatgagaagctccctgaagacatctctgagaggtatgtcttcctcctggaccccatgctggcaactggaggctctgcaatcatggccactgaggtgctcatcaagaggggagtcaagcctgagaggatctacttcctcaacctcatctgctcaaaggagggcattgagaagtaccatgctgccttccctgaagtgaggattgtcactggggctctggacaggggcctggatgagaacaagtacctggtccctggcctgggagactttggggacagatactactgtgtctaa

SEQ ID NO: 57 - protein, 90 aa, synthetic construct
MVTGGMASKWDQKGMDIAYEEAALGYKEGGVPIGGCLINNKDGSVLGRGHNMRFQKGSATLHGEISTLENCGRLEGKVYKDTTLYTTLSP

SEQ ID NO: 58 - DNA, 1022 bp, synthetic construct
  source 1..1022: mol_type = other DNA
  CDS 1..1022: protein_id = 59; translation = DIAYEEAALGYKEGGVPIGGCLINNKDGSVLGRGHNMRFQKGSATLHGEISTLENCGRLEGKVYKDTTLYTTLSPCDMCTGAIIMYGIPRCVVGENVNFKSKGEKYLQTRGHEVVVVDDERCKKIMKQFIDERPQDWFEDIGEASEPFKNVYLLPQTNQLLGLYTIIRNKNTTRPDFIFYSDRIIRLLVEEGLNHLPVQKQIVETDTNENFEGVSFMGKICGVSIVRAGESMEQGLRDCCRSVRIGKILIQRDEETALPKLFYEKLPEDISERYVFLLDPMLATGGSAIMATEVLIKRGVKPERIYFLNLICSKEGIEKYHAAFPEVRIVTGALDRGLDE
gacattgcctatgaggaggctgctctgggctacaaggagggaggggtcccaattggtggctgcctcatcaacaacaaggatggcagtgtcctgggcaggggccacaacatgaggttccagaagggcagtgccaccctgcatggggagatcagcaccctggagaactgtggcaggctggagggcaaggtctacaaggacaccactctgtacaccaccctcagcccttgtgacatgtgcacaggggccatcatcatgtatggcattcccaggtgtgtggtgggagagaatgtcaacttcaagtcaaaaggagagaagtacctccagaccaggggccatgaggtggttgtggtggatgatgagaggtgcaagaagattatgaagcagttcattgatgagagaccccaggactggtttgaggacattggggaggcctctgagcccttcaagaatgtgtacctcctcccccagaccaaccaactcctgggactctacaccatcatcaggaacaagaacaccaccaggccagacttcatcttctacagtgacaggatcatcaggctcctggtggaggagggcctcaaccacctccctgtgcagaagcagattgtggagactgacaccaatgagaactttgagggagtgtctttcatgggcaagatttgtggggtgtccattgtgagggctggggagagcatggagcagggcctgagggactgttgcaggagtgtgaggattggcaagatcctgatccagagggatgaggagactgccctgcccaagctgttctatgagaagctccctgaagacatctctgagaggtatgtcttcctcctggaccccatgctggcaactggaggctctgcaatcatggccactgaggtgctcatcaagaggggagtcaagcctgagaggatctacttcctcaacctcatctgctcaaaggagggcattgagaagtaccatgctgccttccctgaagtgaggattgtcactggggctctggacaggggcctggatgagaa

SEQ ID NO: 59 - protein, 340 aa, synthetic construct
DIAYEEAALGYKEGGVPIGGCLINNKDGSVLGRGHNMRFQKGSATLHGEISTLENCGRLEGKVYKDTTLYTTLSPCDMCTGAIIMYGIPRCVVGENVNFKSKGEKYLQTRGHEVVVVDDERCKKIMKQFIDERPQDWFEDIGEASEPFKNVYLLPQTNQLLGLYTIIRNKNTTRPDFIFYSDRIIRLLVEEGLNHLPVQKQIVETDTNENFEGVSFMGKICGVSIVRAGESMEQGLRDCCRSVRIGKILIQRDEETALPKLFYEKLPEDISERYVFLLDPMLATGGSAIMATEVLIKRGVKPERIYFLNLICSKEGIEKYHAAFPEVRIVTGALDRGLDE

SEQ ID NO: 60 - DNA, 23 bp, synthetic construct
  source 1..23: mol_type = other DNA
taatacgactcactataggctag

SEQ ID NO: 61 - DNA, 41 bp, synthetic construct
  source 1..41: mol_type = other DNA
gccgccccgactctagtcactccccaatgtcctcaaaccag

SEQ ID NO: 62 - DNA, 46 bp, synthetic construct
  source 1..46: mol_type = other DNA
ctagcctcgagaccggtcaccatgtcctctgagcccttcaagaatg

SEQ ID NO: 63 - DNA, 20 bp, synthetic construct
  source 1..20: mol_type = other DNA
gagtgcaccatacgcggatc

SEQ ID NO: 64 - DNA, 46 bp, synthetic construct
  source 1..46: mol_type = other DNA
attaccctgttatccctacgcgtcaagggctgagggtggtgtacag

SEQ ID NO: 65 - DNA, 46 bp, synthetic construct
  source 1..46: mol_type = other DNA
gcgtagggataacagggtaatgcatatggcattcccaggtgtgtgg

SEQ ID NO: 66 - DNA, 39 bp, synthetic construct
  source 1..39: mol_type = other DNA
catggctcgacagatctgacattgcctatgaggaggctg

SEQ ID NO: 67 - DNA, 38 bp, synthetic construct
  source 1..38: mol_type = other DNA
ggccaatattgaagatcttctcatccaggcccctgtcc

SEQ ID NO: 68 - DNA, 720 bp, synthetic construct
  source 1..720: mol_type = other DNA
  CDS 1..720: protein_id = 69; translation = MVSKGEELFTGVVPILVELDGDVNGHKFSVSGEGEGDATYGKLTLKFICTTGKLPVPWPTLVTTLSWGVQCFARYPDHMKQHDFFKSAMPEGYVQERTIFFKDDGNYKTRAEVKFEGDTLVNRIELKGIDFKEDGNILGHKLEYNYFSDNVYITADKQKNGIKANFKIRHNIEDGGVQLADHYQQNTPIGDGPVLLPDNHYLSTQSKLSKDPNEKRDHMVLLEFVTAAGITLGMDELYK
atggtgagcaagggcgaggagctgttcaccggggtggtgcccatcctggtcgagctggacggcgacgtaaacggccacaagttcagcgtgtccggcgagggcgagggcgatgccacctacggcaagctgaccctgaagttcatctgcaccaccggcaagctgcccgtgccctggcccaccctcgtgaccaccctgtcctggggcgtgcagtgcttcgcccgctaccccgaccacatgaagcagcacgacttcttcaagtccgccatgcccgaaggctacgtccaggagcgcaccatcttcttcaaggacgacggcaactacaagacccgcgccgaggtgaagttcgagggcgacaccctggtgaaccgcatcgagctgaagggcatcgacttcaaggaggacggcaacatcctggggcacaagctggagtacaactactttagcgacaacgtctatatcaccgccgacaagcagaagaacggcatcaaggccaacttcaagatccgccacaacatcgaggacggcggcgtgcagctcgccgaccactaccagcagaacacccccatcggcgacggccccgtgctgctgcccgacaaccactacctgagcacccagtccaagctgagcaaagaccccaacgagaagcgcgatcacatggtcctgctggagttcgtgaccgccgccgggatcaccctgggcatggacgagctgtacaagtag

SEQ ID NO: 69 - protein, 239 aa, synthetic construct
MVSKGEELFTGVVPILVELDGDVNGHKFSVSGEGEGDATYGKLTLKFICTTGKLPVPWPTLVTTLSWGVQCFARYPDHMKQHDFFKSAMPEGYVQERTIFFKDDGNYKTRAEVKFEGDTLVNRIELKGIDFKEDGNILGHKLEYNYFSDNVYITADKQKNGIKANFKIRHNIEDGGVQLADHYQQNTPIGDGPVLLPDNHYLSTQSKLSKDPNEKRDHMVLLEFVTAAGITLGMDELYK

SEQ ID NO: 70 - DNA, 1200 bp, synthetic construct
  source 1..1200: mol_type = other DNA
  CDS 1..1200: protein_id = 71; translation = MVSKGEELFTGVVPILVELDGDVNGHKFSVSGEGEGDATYGKLTLKFICTTGKLPVPWPTLVTTLSWGVQCFARYPDHMKQHDFFKSAMPEGYVQERTIFFKDDGNYKTRAEVKFEGDTLVNRIELKGIDFKEDGNILGHKLEYNYFSDNVYITADKQKNGIKANFKIRHNIEDGGVQLADHYQQNTPIGDGPVLLPDNHYLSTQSKLSKDPNEKRDHMVLLEFVTAAGLHTLEDFVGDWRQTAGYNLDQVLEQGGVSSLFQNLGVSVTPIQRIVLSGENGLKIDIHVIIPYEGLSGDQMGQIEKIFKVVYPVDDHHFKVILHYGTLVIDGVTPNMIDYFGRPYEGIAVFDGKKITVTGTLWNGNKIIDERLINPDGSLLFRVTINGVTGWRLCERILA
atggtgagcaagggcgaggagctgttcaccggggtggtgcccatcctggtcgagctggacggcgacgtaaacggccacaagttcagcgtgtccggcgagggcgagggcgatgccacctacggcaagctgaccctgaagttcatctgcaccaccggcaagctgcccgtgccctggcccaccctcgtgaccaccctgtcctggggcgtgcagtgcttcgcccgctaccccgaccacatgaagcagcacgacttcttcaagtccgccatgcccgaaggctacgtccaggagcgcaccatcttcttcaaggacgacggcaactacaagacccgcgccgaggtgaagttcgagggcgacaccctggtgaaccgcatcgagctgaagggcatcgacttcaaggaggacggcaacatcctggggcacaagctggagtacaactactttagcgacaacgtctatatcaccgccgacaagcagaagaacggcatcaaggccaacttcaagatccgccacaacatcgaggacggcggcgtgcagctcgccgaccactaccagcagaacacccccatcggcgacggccccgtgctgctgcccgacaaccactacctgagcacccagtccaagctgagcaaagaccccaacgagaagcgcgatcacatggtcctgctggagttcgtgaccgccgccgggttgcatacactcgaagatttcgttggggactggcgacagacagccggctacaacctggaccaagtccttgaacagggaggtgtgtccagtttgtttcagaatctcggggtgtccgtaactccgatccaaaggattgtcctgagcggtgaaaatgggctgaagatcgacatccatgtcatcatcccgtatgaaggtctgagcggcgaccaaatgggccagatcgaaaaaatttttaaggtggtgtaccctgtggatgatcatcactttaaggtgatcctgcactatggcacactggtaatcgacggggttacgccgaacatgatcgactatttcggacggccgtatgaaggcatcgccgtgttcgacggcaaaaagatcactgtaacagggaccctgtggaacggcaacaaaattatcgacgagcgcctgatcaaccccgacggctccctgctgttccgagtaaccatcaacggagtgaccggctggcggctgtgcgaacgcattctggcgtaa

SEQ ID NO: 71 - protein, 399 aa, synthetic construct
MVSKGEELFTGVVPILVELDGDVNGHKFSVSGEGEGDATYGKLTLKFICTTGKLPVPWPTLVTTLSWGVQCFARYPDHMKQHDFFKSAMPEGYVQERTIFFKDDGNYKTRAEVKFEGDTLVNRIELKGIDFKEDGNILGHKLEYNYFSDNVYITADKQKNGIKANFKIRHNIEDGGVQLADHYQQNTPIGDGPVLLPDNHYLSTQSKLSKDPNEKRDHMVLLEFVTAAGLHTLEDFVGDWRQTAGYNLDQVLEQGGVSSLFQNLGVSVTPIQRIVLSGENGLKIDIHVIIPYEGLSGDQMGQIEKIFKVVYPVDDHHFKVILHYGTLVIDGVTPNMIDYFGRPYEGIAVFDGKKITVTGTLWNGNKIIDERLINPDGSLLFRVTINGVTGWRLCERILA

SEQ ID NO: 72 - DNA, 1080 bp, synthetic construct
  source 1..1080: mol_type = other DNA
  CDS 1..603: protein_id = 73; translation = MVSKGEELFTGVVPILVELDGDVNGHKFSVSGEGEGDATYGKLTLKFICTTGKLPVPWPTLVTTLSWGVQCFARYPDHMKQHDFFKSAMPEGYVQERTIFFKDDGNYKTRAEVKFEGDTLVNRIELKGIDFKEDGNILGHKLEYNYFSDNVYITADKQKNGIKANFKIRHNIEDGGVQLADHYQQNTPIGDGPVLLPDNH
atggtgagcaagggcgaggagctgttcaccggggtggtgcccatcctggtcgagctggacggcgacgtaaacggccacaagttcagcgtgtccggcgagggcgagggcgatgccacctacggcaagctgaccctgaagttcatctgcaccaccggcaagctgcccgtgccctggcccaccctcgtgaccaccctgtcctggggcgtgcagtgcttcgcccgctaccccgaccacatgaagcagcacgacttcttcaagtccgccatgcccgaaggctacgtccaggagcgcaccatcttcttcaaggacgacggcaactacaagacccgcgccgaggtgaagttcgagggcgacaccctggtgaaccgcatcgagctgaagggcatcgacttcaaggaggacggcaacatcctggggcacaagctggagtacaactactttagcgacaacgtctatatcaccgccgacaagcagaagaacggcatcaaggccaacttcaagatccgccacaacatcgaggacggcggcgtgcagctcgccgaccactaccagcagaacacccccatcggcgacggccccgtgctgctgcccgacaaccactgaattctagggataacagggtaatgcatagtccttgaacagggaggtgtgtccagtttgtttcagaatctcggggtgtccgtaactccgatccaaaggattgtcctgagcggtgaaaatgggctgaagatcgacatccatgtcatcatcccgtatgaaggtctgagcggcgaccaaatgggccagatcgaaaaaatttttaaggtggtgtaccctgtggatgatcatcactttaaggtgatcctgcactatggcacactggtaatcgacggggttacgccgaacatgatcgactatttcggacggccgtatgaaggcatcgccgtgttcgacggcaaaaagatcactgtaacagggaccctgtggaacggcaacaaaattatcgacgagcgcctgatcaaccccgacggctccctgctgttccgagtaaccatcaacggagtgaccggctggcggctgtgcgaacgcattctggcgtaa

SEQ ID NO: 73 - protein, 200 aa, synthetic construct
MVSKGEELFTGVVPILVELDGDVNGHKFSVSGEGEGDATYGKLTLKFICTTGKLPVPWPTLVTTLSWGVQCFARYPDHMKQHDFFKSAMPEGYVQERTIFFKDDGNYKTRAEVKFEGDTLVNRIELKGIDFKEDGNILGHKLEYNYFSDNVYITADKQKNGIKANFKIRHNIEDGGVQLADHYQQNTPIGDGPVLLPDNH

SEQ ID NO: 74 - protein, 6 aa, synthetic construct
ILGITG

SEQ ID NO: 75 - protein, 151 aa, synthetic construct
CIVLEQGGVSSLFQNLGVSVTPIQRIVLSGENGLKIDIHVIIPYEGLSGDQMGQIEKIFKVVYPVDDHHFKVILHYGTLVIDGVTPNMIDYFGRPYEGIAVFDGKKITVTGTLWNGNKIIDERLINPDGSLLFRVTINGVTGWRLCERILA

SEQ ID NO: 76 - DNA, 944 bp, synthetic construct
  source 1..944: mol_type = other DNA
  CDS 3..944: protein_id = 77; translation = FARYPDHMKQHDFFKSAMPEGYVQERTIFFKDDGNYKTRAEVKFEGDTLVNRIELKGIDFKEDGNILGHKLEYNYFSDNVYITADKQKNGIKANFKIRHNIEDGGVQLADHYQQNTPIGDGPVLLPDNHYLSTQSKLSKDPNEKRDHMVLLEFVTAAGLHTLEDFVGDWRQTAGYNLDQVLEQGGVSSLFQNLGVSVTPIQRIVLSGENGLKIDIHVIIPYEGLSGDQMGQIEKIFKVVYPVDDHHFKVILHYGTLVIDGVTPNMIDYFGRPYEGIAVFDGKKITVTGTLWNGNKIIDERLINPDGSLLFRVTI
gcttcgcccgctaccccgaccacatgaagcagcacgacttcttcaagtccgccatgcccgaaggctacgtccaggagcgcaccatcttcttcaaggacgacggcaactacaagacccgcgccgaggtgaagttcgagggcgacaccctggtgaaccgcatcgagctgaagggcatcgacttcaaggaggacggcaacatcctggggcacaagctggagtacaactactttagcgacaacgtctatatcaccgccgacaagcagaagaacggcatcaaggccaacttcaagatccgccacaacatcgaggacggcggcgtgcagctcgccgaccactaccagcagaacacccccatcggcgacggccccgtgctgctgcccgacaaccactacctgagcacccagtccaagctgagcaaagaccccaacgagaagcgcgatcacatggtcctgctggagttcgtgaccgccgccgggttgcatacactcgaagatttcgttggggactggcgacagacagccggctacaacctggaccaagtccttgaacagggaggtgtgtccagtttgtttcagaatctcggggtgtccgtaactccgatccaaaggattgtcctgagcggtgaaaatgggctgaagatcgacatccatgtcatcatcccgtatgaaggtctgagcggcgaccaaatgggccagatcgaaaaaatttttaaggtggtgtaccctgtggatgatcatcactttaaggtgatcctgcactatggcacactggtaatcgacggggttacgccgaacatgatcgactatttcggacggccgtatgaaggcatcgccgtgttcgacggcaaaaagatcactgtaacagggaccctgtggaacggcaacaaaattatcgacgagcgcctgatcaaccccgacggctccctgctgttccgagtaaccatc

SEQ ID NO: 77 - protein, 314 aa, synthetic construct
FARYPDHMKQHDFFKSAMPEGYVQERTIFFKDDGNYKTRAEVKFEGDTLVNRIELKGIDFKEDGNILGHKLEYNYFSDNVYITADKQKNGIKANFKIRHNIEDGGVQLADHYQQNTPIGDGPVLLPDNHYLSTQSKLSKDPNEKRDHMVLLEFVTAAGLHTLEDFVGDWRQTAGYNLDQVLEQGGVSSLFQNLGVSVTPIQRIVLSGENGLKIDIHVIIPYEGLSGDQMGQIEKIFKVVYPVDDHHFKVILHYGTLVIDGVTPNMIDYFGRPYEGIAVFDGKKITVTGTLWNGNKIIDERLINPDGSLLFRVTI

SEQ ID NO: 78 - DNA, 45 bp, synthetic construct
  source 1..45: mol_type = other DNA
ttaccctgttatccctagaattcagtggttgtcgggcagcagcac

SEQ ID NO: 79 - DNA, 46 bp, synthetic construct
  source 1..46: mol_type = other DNA
tctagggataacagggtaatgcatagtccttgaacagggaggtgtg

SEQ ID NO: 80 - DNA, 39 bp, synthetic construct
  source 1..39: mol_type = other DNA
acatggctcgacagatctgcttcgcccgctaccccgacc

SEQ ID NO: 81 - DNA, 40 bp, synthetic construct
  source 1..40: mol_type = other DNA
ggccaatattgaagatctgatggttactcggaacagcagg

SEQ ID NO: 82 - RNA, 477 nt, Saccharomyces cerevisiae
  source 1..477: mol_type = mRNA
atggtgacagggggaatggcaagcaagtgggatcagaagggtatggacattgcctatgaggaggcggccttaggttacaaagagggtggtgttcctattggcggatgtcttatcaataacaaagacggaagtgttctcggtcgtggtcacaacatgagatttcaaaagggatccgccacactacatggtgagatctccactttggaaaactgtgggagattagagggcaaagtgtacaaagataccactttgtatacgacgctgtctccatgcgacatgtgtacaggtgccatcatcatgtatggtattccacgctgtgttgtcggtgagaacgttaatttcaaaagtaagggcgagaaatatttacaaactagaggtcacgaggttgttgttgttgacgatgagaggtgtaaaaagatcatgaaacaatttatcgatgaaagacctcaggattggtttgaagatattggtgagtag

SEQ ID NO: 83 - RNA, 651 nt, Saccharomyces cerevisiae
  source 1..651: mol_type = mRNA
atgtcttcggaaccatttaagaacgtctacttgctacctcaaacaaaccaattgctgggtttgtacaccatcatcagaaataagaatacaactagacctgatttcattttctactccgatagaatcatcagattgttggttgaagaaggtttgaaccatctacctgtgcaaaagcaaattgtggaaactgacaccaacgaaaacttcgaaggtgtctcattcatgggtaaaatctgtggtgtttccattgtcagagctggtgaatcgatggagcaaggattaagagactgttgtaggtctgtgcgtatcggtaaaattttaattcaaagggacgaggagactgctttaccaaagttattctacgaaaaattaccagaggatatatctgaaaggtatgtcttcctattagacccaatgctggccaccggtggtagtgctatcatggctacagaagtcttgattaagagaggtgttaagccagagagaatttacttcttaaacctaatctgtagtaaggaagggattgaaaaataccatgccgccttcccagaggtcagaattgttactggtgccctcgacagaggtctagatgaaaacaagtatctagttccagggttgggtgactttggtgacagatactactgtgtttaa

SEQ ID NO: 84 - DNA, 1284 bp, Escherichia coli
  source 1..1284: mol_type = other DNA
  CDS 1..1284: protein_id = 85; translation = MSNNALQTIINARLPGEEGLWQIHLQDGKISAIDAQSGVMPITENSLDAEQGLVIPPFVEPHIHLDTTQTAGQPNWNQSGTLFEGIERWAERKALLTHDDVKQRAWQTLKWQIANGIQHVRTHVDVSDATLTALKAMLEVKQEVAPWIDLQIVAFPQEGILSYPNGEALLEEALRLGADVVGAIPHFEFTREYGVESLHKTFALAQKYDRLIDVHCDEIDDEQSRFVETVAALAHHEGMGARVTASHTTAMHSYNGAYTSRLFRLLKMSGINFVANPLVNIHLQGRFDTYPKRRGITRVKEMLESGINVCFGHDDVFDPWYPLGTANMLQVLHMGLHVCQLMGYGQINDGLNLITHHSARTLNLQDYGIAAGNSANLIILPAENGFDALRRQVPVRYSVRGGKVIASTQPAQTTVYLEQPEAIDYKR
atgtcgaataacgctttacaaacaattattaacgcccggttaccaggcgaagaggggctgtggcagattcatctgcaggacggaaaaatcagcgccattgatgcgcaatccggcgtgatgcccataactgaaaacagcctggatgccgaacaaggtttagttataccgccgtttgtggagccacatattcacctggacaccacgcaaaccgccggacaaccgaactggaatcagtccggcacgctgtttgaaggcattgaacgctgggccgagcgcaaagcgttattaacccatgacgatgtgaaacaacgcgcatggcaaacgctgaaatggcagattgccaacggcattcagcatgtgcgtacccatgtcgatgtttcggatgcaacgctaactgcgctgaaagcaatgctggaagtgaagcaggaagtcgcgccgtggattgatctgcaaatcgtcgccttccctcaggaagggattttgtcgtatcccaacggtgaagcgttgctggaagaggcgttacgcttaggggcagatgtagtgggggcgattccgcattttgaatttacccgtgaatacggcgtggagtcgctgcataaaaccttcgccctggcgcaaaaatacgaccgtctcatcgacgttcactgtgatgagatcgatgacgagcagtcgcgctttgtcgaaaccgttgctgccctggcgcaccatgaaggcatgggcgcgcgagtcaccgccagccacaccacggcaatgcactcctataacggggcgtatacctcacgcctgttccgcttgctgaaaatgtccggtattaactttgtcgccaacccgctggtcaatattcatctgcaaggacgtttcgatacgtatccaaaacgtcgcggcatcacgcgcgttaaagagatgctggagtccggcattaacgtctgctttggtcacgatgatgtcttcgatccgtggtatccgctgggaacggcgaatatgctgcaagtgctgcatatggggctgcatgtttgccagttgatgggctacgggcagattaacgatggcctgaatttaatcacccaccacagcgcaaggacgttgaatttgcaggattacggcattgccgccggaaacagcgccaacctgattatcctgccggctgaaaatgggtttgatgcgctgcgccgtcaggttccggtacgttattcggtacgtggcggcaaggtgattgccagcacacaaccggcacaaaccaccgtatatctggagcagccagaagccatcgattacaaacgttga

SEQ ID NO: 85 - protein, 427 aa, Escherichia coli
MSNNALQTIINARLPGEEGLWQIHLQDGKISAIDAQSGVMPITENSLDAEQGLVIPPFVEPHIHLDTTQTAGQPNWNQSGTLFEGIERWAERKALLTHDDVKQRAWQTLKWQIANGIQHVRTHVDVSDATLTALKAMLEVKQEVAPWIDLQIVAFPQEGILSYPNGEALLEEALRLGADVVGAIPHFEFTREYGVESLHKTFALAQKYDRLIDVHCDEIDDEQSRFVETVAALAHHEGMGARVTASHTTAMHSYNGAYTSRLFRLLKMSGINFVANPLVNIHLQGRFDTYPKRRGITRVKEMLESGINVCFGHDDVFDPWYPLGTANMLQVLHMGLHVCQLMGYGQINDGLNLITHHSARTLNLQDYGIAAGNSANLIILPAENGFDALRRQVPVRYSVRGGKVIASTQPAQTTVYLEQPEAIDYKR

SEQ ID NO: 86 - DNA, 627 bp, Escherichia coli
  source 1..627: mol_type = genomic DNA
  CDS 1..627: protein_id = 87; translation = MKIVEVKHPLVKHKLGLMREQDISTKRFRELASEVGSLLTYEATADLETEKVTIEGWNGPVEIDQIKGKKITVVPILRAGLGMMDGVLENVPSARISVVGMYRNEETLEPVPYFQKLVSNIDERMALIVDPMLATGGSVIATIDLLKKAGCSSIKVLVLVAAPEGIAALEKAHPDVELYTASIDQGLNEHGYIIPGLGDAGDKIFGTK
atgaagatcgtggaagtcaaacacccactcgtcaaacacaagctgggactgatgcgtgagcaagatatcagcaccaagcgctttcgcgaactcgcttccgaagtgggtagcctgctgacttacgaagcgaccgccgacctcgaaacggaaaaagtaactatcgaaggctggaacggcccggtagaaatcgaccagatcaaaggtaagaaaattaccgttgtgccaattctgcgtgcgggtcttggtatgatggacggtgtgctggaaaacgttccgagcgcgcgcatcagcgttgtcggtatgtaccgtaatgaagaaacgctggagccggtaccgtacttccagaaactggtttctaacatcgatgagcgtatggcgctgatcgttgacccaatgctggcaaccggtggttccgttatcgcgaccatcgacctgctgaaaaaagcgggctgcagcagcatcaaagttctggtgctggtagctgcgccagaaggtatcgctgcgctggaaaaagcgcacccggacgtcgaactgtataccgcatcgattgatcagggactgaacgagcacggatacattattccgggcctcggcgatgccggtgacaaaatctttggtacgaaataa

SEQ ID NO: 87 - protein, 208 aa, Escherichia coli
MKIVEVKHPLVKHKLGLMREQDISTKRFRELASEVGSLLTYEATADLETEKVTIEGWNGPVEIDQIKGKKITVVPILRAGLGMMDGVLENVPSARISVVGMYRNEETLEPVPYFQKLVSNIDERMALIVDPMLATGGSVIATIDLLKKAGCSSIKVLVLVAAPEGIAALEKAHPDVELYTASIDQGLNEHGYIIPGLGDAGDKIFGTK

SEQ ID NO: 88 - DNA, 596 bp, synthetic construct
  source 1..596: mol_type = other DNA
aattccgcccctctcccccccccccctctccctcccccccccctaacgttactggccgaagccgcttggaataaggccggtgtgcgtttgtctatatgtgattttccaccatattgccgtcttttggcaatgtgagggcccggaaacctggccctgtcttcttgacgagcattcctaggggtctttcccctctcgccaaaggaatgcaaggtctgttgaatgtcgtgaaggaagcagttcctctggaagcttcttgaagacaaacaacgtctgtagcgaccctttgcaggcagcggaaccccccacctggcgacaggtgcctctgcggccaaaagccacgtgtataagatacacctgcaaaggcggcacaaccccagtgccacgttgtgagttggatagttgtggaaagagtcaaatggctctcctcaagcgtattcaacaaggggctgaaggatgcccagaaggtaccccattgtatgggatctgatctggggcctcggtgcacatgctttacatgtgtttagtcgaggttaaaaaaacgtctaggccccccgaaccacggggacgtggttttcctttgaaaaacacgatgataa

SEQ ID NO: 89 - DNA, 585 bp, synthetic construct
  source 1..585: mol_type = other DNA
gcccctctccctcccccccccctaacgttactggccgaagccgcttggaataaggccggtgtgcgtttgtctatatgttattttccaccatattgccgtcttttggcaatgtgagggcccggaaacctggccctgtcttcttgacgagcattcctaggggtctttcccctctcgccaaaggaatgcaaggtctgttgaatgtcgtgaaggaagcagttcctctggaagcttcttgaagacaaacaacgtctgtagcgaccctttgcaggcagcggaaccccccacctggcgacaggtgcctctgcggccaaaagccacgtgtataagatacacctgcaaaggcggcacaaccccagtgccacgttgtgagttggatagttgtggaaagagtcaaatggctctcctcaagcgtattcaacaaggggctgaaggatgcccagaaggtaccccattgtatgggatctgatctggggcctcggtacacatgctttacatgtgtttagtcgaggttaaaaaaacgtctaggccccccgaaccacggggacgtggttttcctttgaaaaacacgatgataatatggccaca

SEQ ID NO: 90 - DNA, 57 bp, synthetic construct
  source 1..57: mol_type = other DNA
  CDS 1..57: protein_id = 91; translation = ATNFSLLKQAGDVEENPGP
gctactaacttcagcctgctgaagcaggctggagacgtggaggagaaccctggacct

SEQ ID NO: 91 - protein, 19 aa, synthetic construct
ATNFSLLKQAGDVEENPGP

SEQ ID NO: 92 - DNA, 60 bp, synthetic construct
  source 1..60: mol_type = other DNA
  CDS 1..60: protein_id = 93; translation = QCTNYALLKLAGDVESNPGP
caatgtactaactacgctttgttgaaactcgctggcgatgttgaaagtaaccccggtcct

SEQ ID NO: 93 - protein, 20 aa, synthetic construct
QCTNYALLKLAGDVESNPGP

SEQ ID NO: 94 - DNA, 66 bp, synthetic construct
  source 1..66: mol_type = other DNA
  CDS 1..66: protein_id = 95; translation = VKQTLNFDLLKLAGDVESNPGP
gtgaaacagactttgaattttgaccttctcaagttggcgggagacgtggagtccaacccagggccc

SEQ ID NO: 95 - protein, 22 aa, synthetic construct
VKQTLNFDLLKLAGDVESNPGP